European Patent Specification EP 3 202 792 B1, published August 14, 2024. Title: Chimeric antigen receptor containing a Toll-like receptor intracellular domain. Applicant: Shenzhen In Vivo Biomedicine Technology Limited Company. Application 15 900 639.4. The sequence listing filed with the application follows.

SEQUENCE LISTING (17 sequences)

SEQ ID NO: 1 - DNA, 1487 bp, Artificial sequence
  CAR19
gtttaaacgaattcatgcttctcctggtgacaagccttctgctctgtgagttaccacacccagcattcctcctgatcccagacatccagatgacacagactacatcctccctgtctgcctctctgggagacagagtcaccatcagttgcagggcaagtcaggacattagtaaatatttaaattggtatcagcagaaaccagatggaactgttaaactcctgatctaccatacatcaagattacactcaggagtcccatcaaggttcagtggcagtgggtctggaacagattattctctcaccattagcaacctggagcaagaagatattgccacttacttttgccaacagggtaatacgcttccgtacacgttcggaggggggactaagttggaaataacaggctccacctctggatccggcaagcccggatctggcgagggatccaccaagggcgaggtgaaactgcaggagtcaggacctggcctggtggcgccctcacagagcctgtccgtcacatgcactgtctcaggggtctcattacccgactatggtgtaagctggattcgccagcctccacgaaagggtctggagtggctgggagtaatatggggtagtgaaaccacatactataattcagctctcaaatccagactgaccatcatcaaggacaactccaagagccaagttttcttaaaaatgaacagtctgcaaactgatgacacagccatttactactgtgccaaacattattactacggtggtagctatgctatggactactggggtcaaggaacctcagtcaccgtctcctcagcggccgcaattgaagttatgtatcctcctccttacctagacaatgagaagagcaatggaaccattatccatgtgaaagggaaacacctttgtccaagtcccctatttcccggaccttctaagcccttttgggtgctggtggtggttgggggagtcctggcttgctatagcttgctagtaacagtggcctttattattttctgggtgaggagtaagaggagcaggctcctgcacagtgactacatgaacatgactccccgccgccccgggcccacccgcaagcattaccagccctatgccccaccacgcgacttcgcagcctatcgctccagagtgaagttcagcaggagcgcagacgcccccgcgtaccagcagggccagaaccagctctataacgagctcaatctaggacgaagagaggagtacgatgttttggacaagagacgtggccgggaccctgagatggggggaaagccgagaaggaagaaccctcaggaaggcctgtacaatgaactgcagaaagataagatggcggaggcctacagtgagattgggatgaaaggcgagcgccggaggggcaaggggcacgatggcctttaccagggtctcagtacagccaccaaggacacctacgacgcccttcacatgcaggccctgccccctcgcactagt

SEQ ID NO: 2 - DNA, 21 bp, Artificial sequence
  TLR1/2 overlapA
gcggccgcaattgaagttatg

SEQ ID NO: 3 - DNA, 38 bp, Artificial sequence
  TLR1 overlap B1
catgcaggccctgccccctcgcaacatacccttagaag

SEQ ID NO: 4 - DNA, 38 bp, Artificial sequence
  TLR1 overlap B2
cttctaagggtatgttgcgagggggcagggcctgcatg

SEQ ID NO: 5 - DNA, 28 bp, Artificial sequence
  TLR1 overlap C
actagttttctttgcttgctctgtcagc

SEQ ID NO: 6 - DNA, 42 bp, Artificial sequence
  TLR2 overlap B1
catgcaggccctgccccctcgccaggccaaaaggaagcccag

SEQ ID NO: 7 - DNA, 42 bp, Artificial sequence
  TLR2 overlap B2
ctgggcttccttttggcctggcgagggggcagggcctgcatg

SEQ ID NO: 8 - DNA, 27 bp, Artificial sequence
  TLR2 overlap C
actagtggactttatcgcagctctcag

SEQ ID NO: 9 - DNA, 1158 bp, Artificial sequence
  28ZT1
gcggccgcaattgaagttatgtatcctcctccttacctagacaatgagaagagcaatggaaccattatccatgtgaaagggaaacacctttgtccaagtcccctatttcccggaccttctaagcccttttgggtgctggtggtggttgggggagtcctggcttgctatagcttgctagtaacagtggcctttattattttctgggtgaggagtaagaggagcaggctcctgcacagtgactacatgaacatgactccccgccgccccgggcccacccgcaagcattaccagccctatgccccaccacgcgacttcgcagcctatcgctccagagtgaagttcagcaggagcgcagacgcccccgcgtaccagcagggccagaaccagctctataacgagctcaatctaggacgaagagaggagtacgatgttttggacaagagacgtggccgggaccctgagatggggggaaagccgagaaggaagaaccctcaggaaggcctgtacaatgaactgcagaaagataagatggcggaggcctacagtgagattgggatgaaaggcgagcgccggaggggcaaggggcacgatggcctttaccagggtctcagtacagccaccaaggacacctacgacgcccttcacatgcaggccctgccccctcgcaacatacccttagaagaactccaaagaaatctccagtttcatgcatttatttcatatagtgggcacgattctttctgggtgaagaatgaattattgccaaacctagagaaagaaggtatgcagatttgccttcatgagagaaactttgttcctggcaagagcattgtggaaaatatcatcacctgcattgagaagagttacaagtccatctttgttttgtctcccaactttgtccagagtgaatggtgccattatgaactctactttgcccatcacaatctctttcatgaaggatctaatagcttaatcctgatcttgctggaacccattccgcagtactccattcctagcagttatcacaagctcaaaagtctcatggccaggaggacttatttggaatggcccaaggaaaagagcaaacgtggccttttttgggctaacttaagggcagccattaatattaagctgacagagcaagcaaagaaaactagt

SEQ ID NO: 10 - DNA, 1149 bp, Artificial sequence
  28ZT2
gcggccgcaattgaagttatgtatcctcctccttacctagacaatgagaagagcaatggaaccattatccatgtgaaagggaaacacctttgtccaagtcccctatttcccggaccttctaagcccttttgggtgctggtggtggttgggggagtcctggcttgctatagcttgctagtaacagtggcctttattattttctgggtgaggagtaagaggagcaggctcctgcacagtgactacatgaacatgactccccgccgccccgggcccacccgcaagcattaccagccctatgccccaccacgcgacttcgcagcctatcgctccagagtgaagttcagcaggagcgcagacgcccccgcgtaccagcagggccagaaccagctctataacgagctcaatctaggacgaagagaggagtacgatgttttggacaagagacgtggccgggaccctgagatggggggaaagccgagaaggaagaaccctcaggaaggcctgtacaatgaactgcagaaagataagatggcggaggcctacagtgagattgggatgaaaggcgagcgccggaggggcaaggggcacgatggcctttaccagggtctcagtacagccaccaaggacacctacgacgcccttcacatgcaggccctgccccctcgccaggccaaaaggaagcccaggaaagctcccagcaggaacatctgctatgatgcatttgtttcttacagtgagcgggatgcctactgggtggagaaccttatggtccaggagctggagaacttcaatccccccttcaagttgtgtcttcataagcgggacttcattcctggcaagtggatcattgacaatatcattgactccattgaaaagagccacaaaactgtctttgtgctttctgaaaactttgtgaagagtgagtggtgcaagtatgaactggacttctcccatttccgtctttttgatgagaacaatgatgctgccattctcattcttctggagcccattgagaaaaaagccattccccagcgcttctgcaagctgcggaagataatgaacaccaagacctacctggagtggcccatggacgaggctcagcgggaaggattttgggtaaatctgagagctgcgataaagtccactagt

SEQ ID NO: 11 - DNA, 486 bp, Artificial sequence
  TLR1 TIR domain
aacatacccttagaagaactccaaagaaatctccagtttcatgcatttatttcatatagtgggcacgattctttctgggtgaagaatgaattattgccaaacctagagaaagaaggtatgcagatttgccttcatgagagaaactttgttcctggcaagagcattgtggaaaatatcatcacctgcattgagaagagttacaagtccatctttgttttgtctcccaactttgtccagagtgaatggtgccattatgaactctactttgcccatcacaatctctttcatgaaggatctaatagcttaatcctgatcttgctggaacccattccgcagtactccattcctagcagttatcacaagctcaaaagtctcatggccaggaggacttatttggaatggcccaaggaaaagagcaaacgtggccttttttgggctaacttaagggcagccattaatattaagctgacagagcaagcaaagaaa

SEQ ID NO: 12 - DNA, 477 bp, Artificial sequence
  TLR2 TIR domain
caggccaaaaggaagcccaggaaagctcccagcaggaacatctgctatgatgcatttgtttcttacagtgagcgggatgcctactgggtggagaaccttatggtccaggagctggagaacttcaatccccccttcaagttgtgtcttcataagcgggacttcattcctggcaagtggatcattgacaatatcattgactccattgaaaagagccacaaaactgtctttgtgctttctgaaaactttgtgaagagtgagtggtgcaagtatgaactggacttctcccatttccgtctttttgatgagaacaatgatgctgccattctcattcttctggagcccattgagaaaaaagccattccccagcgcttctgcaagctgcggaagataatgaacaccaagacctacctggagtggcccatggacgaggctcagcgggaaggattttgggtaaatctgagagctgcgataaagtcc

SEQ ID NO: 13 - protein, 162 aa, Artificial sequence
  TIR1 amino acid sequence
NIPLEELQRNLQFHAFISYSGHDSFWVKNELLPNLEKEGMQICLHERNFVPGKSIVENIITCIEKSYKSIFVLSPNFVQSEWCHYELYFAHHNLFHEGSNSLILILLEPIPQYSIPSSYHKLKSLMARRTYLEWPKEKSKRGLFWANLRAAINIKLTEQAKK

SEQ ID NO: 14 - protein, 159 aa, Artificial sequence
  TIR2 amino acid sequence
QAKRKPRKAPSRNICYDAFVSYSERDAYWVENLMVQELENFNPPFKLCLHKRDFIPGKWIIDNIIDSIEKSHKTVFVLSENFVKSEWCKYELDFSHFRLFDENNDAAILILLEPIEKKAIPQRFCKLRKIMNTKTYLEWPMDEAQREGFWVNLRAAIKS

SEQ ID NO: 15 - DNA, 803 bp, Artificial sequence
  CAR19 ScFv sequence
atgcttctcctggtgacaagccttctgctctgtgagttaccacacccagcattcctcctgatcccagacatccagatgacacagactacatcctccctgtctgcctctctgggagacagagtcaccatcagttgcagggcaagtcaggacattagtaaatatttaaattggtatcagcagaaaccagatggaactgttaaactcctgatctaccatacatcaagattacactcaggagtcccatcaaggttcagtggcagtgggtctggaacagattattctctcaccattagcaacctggagcaagaagatattgccacttacttttgccaacagggtaatacgcttccgtacacgttcggaggggggactaagttggaaataacaggctccacctctggatccggcaagcccggatctggcgagggatccaccaagggcgaggtgaaactgcaggagtcaggacctggcctggtggcgccctcacagagcctgtccgtcacatgcactgtctcaggggtctcattacccgactatggtgtaagctggattcgccagcctccacgaaagggtctggagtggctgggagtaatatggggtagtgaaaccacatactataattcagctctcaaatccagactgaccatcatcaaggacaactccaagagccaagttttcttaaaaatgaacagtctgcaaactgatgacacagccatttactactgtgccaaacattattactacggtggtagctatgctatggactactggggtcaaggaacctcagtcaccgtctcctcagc

SEQ ID NO: 16 - DNA, 852 bp, Artificial sequence
  CAR22 ScFv sequence
atggttctgctggtcacatcactgctcctctgtgaactgcctcatcctgcctttctgctcattcccgacactgaagtccagctcgtggaatctggagggggcctggtgaaacctgggggatctctcaaactgtcttgtgccgcttctggctttgcttttagcatctacgacatgtcctgggtccggcagacacctgaaaaacgcctggagtgggtcgcctacatttctagtgggggcggaacatactaccccgataccgtgaagggacgctttacaatttctagggataacgccaaaaacaccctgtacctccagatgtcatccctgaaatctgaggatactgccatgtactactgtgctaggcattctggctacggaacacattggggagtgctcttcgcttactggggccaggggactctcgtcactgtctctgctggcgggggaggctctggcggaggcggatccggaggcggagggagtgatattcagatgactcagaccacctcttctctgtccgcttctctgggcgatagagtgacaatctcctgtcgggcatcacaggatattagcaattacctgaactggtaccagcagaaacccgatggaaccgtcaaactgctcatctactacacctccatcctccactctggcgtgccatctcgattttctggatctggctctggaaccgactactctctcacaatctccaacctggaacaggaggattttgccacctacttttgtcagcagggcaatactctgccttggacctttgggggcggaaccaaactggaaatcaaggccaaaacaaccccaccttccgtgtacggccgagtgaaagaccctaag

SEQ ID NO: 17 - DNA, 867 bp, Artificial sequence
  CARMeso ScFv sequence
atgcttctcctggtgacaagccttctgctctgtgagttaccacacccagcattcctcctgatcccaagccaggtacagctgcagcagtcaggtccaggactcgtgacgccctcgcagaccctctcactcacctgtgccatctccggggacagtgtctctagcaacagtgctacttggaactggatcaggcagtccccatcgagaggccttgagtggctgggaaggacatactacaggtccaagtggtataacgactatgcagtatctgtgaaaagtcgaatgagcatcaacccagacacatccaagaaccagttctccctgcagctgaactctgtgactcccgaggacacggctgtgtattactgtgcaagaggaatgatgacttactattacggtatggacgtctggggccaagggaccacggtcaccgtctcctcaggaattctaggatccggtggcggtggcagcggcggtggtggttccggaggcggcggttctcagcctgtgctgactcagtcgtcttccctctctgcatctcctggagcatcagccagtctcacctgcaccttgcgcagtggcatcaatgttggtccctacaggatatactggtaccagcagaagccagggagtcctccccagtatctcctgaactacaaatcagactcagataagcagcagggctctggagtccccagccgcttctctggatccaaagatgcttcggccaatgcaggggttttactcatctctgggctccggtctgaggatgaggctgactattactgtatgatttggcacagcagcgctgctgtgttcggaggaggcacccaactgaccgtcctctccggaattctagaacaacagggt